European Patent Specification EP 3 673 039 B1, published March 19, 2025. Title: PRODUCTION OF BREWER'S WORT HAVING INCREASE FERMENTABLE SUGARS FOR FERMENTATION. Applicant: DUPONT NUTRITION BIOSCIENCES APS. The sequence listing filed with the application follows.

SEQUENCE LISTING (5 sequences)

SEQ ID NO: 1 - protein, 561 aa, Fusarium verticillioides
SPGGSSLDRFISKEADISIKGVLANIGADGKRAQGAAPGAVVASPSRTDPDYWYTWTRDSALTYKVLVERFIHGDKSLQRKIDEYVSAQAKLQGVTNPSGGPESGGLGEPKFHVNLTAFTGSWGRPQRDGPPLRATALTLYANWLVSHGDRSKAVNKVWPVIEKDLAYTVKFWNRTGYDLWEEVNGSSFFTLSASHRALVEGAALAKKLGKSCSDCATNAPRVLCFMQSFWTGSYIDSNINVNDGRKGLDANSILSSIHTFDPSSKCTDSTFQPCSSRALANHKEVVDSFRSIYGVNKNRGKGKAAAVGRYSEDVYYDGNPWYLATLAAAEQLYAAVYQWNKIGSITVDSVSLPFFSDLVPKVSKGTYRKNSKTYKAIIKAVTSYADGFVAVVQTYTPKDGSLAEQFDKSTGTPKSAVHLTWSYASFVGAAERRTGVVPPAWGESNANKVPAVCEAAPACDTTITFNVKNVDVTSDQKVYIVGGITQLSNWAPADGIALEESTSTKGLWTVKVKIPSDTSFEYKYIKKTSDGTVTWESDPNNSAATGSKCGSSSTINDEWR

SEQ ID NO: 2 - protein, 612 aa, Aspergillus fumigatus
APQLSARATGSLDSWLGTETTVALNGILANIGADGAYAKSAKPGIIIASPSTSEPDYYYTWTRDAALVTKVLVDLFRNGNLGLQKVITEYVNSQAYLQTVSNPSGGLASGGLAEPKYNVDMTAFTGAWGRPQRDGPALRATALIDFGNWLIDNGYSSYAVNNIWPIVRNDLSYVSQYWSQSGFDLWEEVNSMSFFTVAVQHRALVEGSTFAKRVGASCSWCDSQAPQILCYMQSFWTGSYINANTGGGRSGKDANTVLASIHTFDPEAGCDDTTFQPCSPRALANHKVYTDSFRSVYAINSGIPQGAAVSAGRYPEDVYYNGNPWFLTTLAAAEQLYDAIYQWKKIGSISITSTSLAFFKDIYSSAAVGTYASSTSTFTDIINAVKTYADGYVSIVQAHAMNNGSLSEQFDKSSGLSLSARDLTWSYAAFLTANMRRNGVVPAPWGAASANSVPSSCSMGSATGTYSTATATSWPSTLTSGSPGSTTTVGTTTSTTSGTAAETACATPTAVAVTFNEIATTTYGENVYIVGSISELGNWDTSKAVALSASKYTSSNNLWYVSVTLPAGTTFEYKYIRKESDGSIVWESDPNRSYTVPAACGVSTATENDTWQ

SEQ ID NO: 3 - protein, 599 aa, Trichoderma reesie
SVDDFISTETPIALNNLLCNVGPDGCRAFGTSAGAVIASPSTIDPDYYYMWTRDSALVFKNLIDRFTETYDAGLQRRIEQYITAQVTLQGLSNPSGSLADGSGLGEPKFELTLKPFTGNWGRPQRDGPALRAIALIGYSKWLINNNYQSTVSNVIWPIVRNDLNYVAQYWNQTGFDLWEEVNGSSFFTVANQHRALVEGATLAATLGQSGSAYSSVAPQVLCFLQRFWVSSGGYVDSNINTNEGRTGKDVNSVLTSIHTFDPNLGCDAGTFQPCSDKALSNLKVVVDSFRSIYGVNKGIPAGAAVAIGRYAEDVYYNGNPWYLATFAAAEQLYDAIYVWKKTGSITVTATSLAFFQELVPGVTAGTYSSSSSTFTNIINAVSTYADGFLSEAAKYVPADGSLAEQFDRNSGTPLSALHLTWSYASFLTATARRAGIVPPSWANSSASTIPSTCSGASVVGSYSRPTATSFPPSQTPKPGVPSGTPYTPLPCATPTSVAVTFHELVSTQFGQTVKVAGNAAALGNWSTSAAVALDAVNYADNHPLWIGTVNLEAGDVVEYKYINVGQDGSVTWESDPNHTYTVPAVACVTQVVKEDTWQS

SEQ ID NO: 4 - protein, 599 aa, Trichoderma reesie
SVDDFISTETPIALNNLLCNVGPDGCRAFGTSAGAVIASPSTIDPDYYYMWTRDSALVFKNLIDRFTETYDAGLQRRIEQYITAQVTLQGLSNPSGSLADGSGLGEPKFELTLKPFTGNWGRPQRDGPALRAIALIGYSKWLINNNYQSTVSNVIWPIVRNDLNYVAQYWNQTGFDLWEEVNGSSFFTVANQHRALVEGATLAATLGQSGSAYSSVAPQVLCFLQRFWVSSGGYVDSNINTNEGRTGKDVNSVLTSIHTFDPNLGCDAGTFQPCSDKALSNLKVVVDSFRSIYGVNKGIPAGAAVAIGRYAEDVYYNGNPWYLATFAAAEQLYDAIYVWKKTGSITVTATSLAFFQELVPGVTAGTYSSSSSTFTNIINAVSTYADGFLSEAAKYVPADGSLAEQFDRNSGTPLSAVHLTWSYASFLTAAARRAGIVPPSWANSSASTIPSTCSGASVVGSYSRPTATSFPPSQTPKPGVPSGTPYTPLPCATPTSVAVTFHELVSTQFGHTVKVAGNAAALGNWSTSAAVALDAVNYRDNHPLWIGTVNLEAGDVVEYKYIIVGQDGSVTWESDPNHTYTVPAVACVTQVVKEDTWQS

SEQ ID NO: 5 - protein, 599 aa, Trichoderma reesie
SVDDFISTETPIALNNLLCNVGPDGCRAFGTSAGAVIASPSTIRPDYYYMWTRDSALVFKNLIDRFTETYDAGLQRRIEQYITAQVTLQGLSNPSGSLADGSGLGEPKFELTLKPFTGNWGRPQRDGPALRAIALIGYSKWLINNNYQSTVSNVIWPIVRNDLNYVAQYWNQTGFDLWEEVNGSSFFTVANQHRALVEGATLAATLGQSGSAYSSVAPQVLCFLQRFWVSSGGYVDSNINTNEGRTGKDVNSVLTSIHTFDPNLGCDAGTFQPCSDKALSNLKVVVDSFRSIYGVNKGIPAGAAVAIGRYAEDVYYNGNPWYLATFAAAEQLYDAIYVWKKTGSITVTATSLAFFQELVPGVTAGTYSSSSSTFTNIINAVSTYADGFLSEAAKYVPADGSLAEQFDRNSGTPLSALHLTWSYASFLTATARRAGIVPPSWANSSASTIPSTCSGASVVGSYSRPTATSFPPSQTPKPGVPSGTPYTPLPCATPTSVAVTFHELVSTQFGQTVKVAGNAAALGNWSTSAAVALDAVNYRDNHPLWIGTVNLEAGDVVEYKYINVGQDGSVTWESDPNHTYTVPAVACVTQVVKEDTWQS